European Patent Specification EP 3 609 433 B1, published February 21, 2024. Title: PROPERTIES AND PARAMETERS OF NOVEL BIODEGRADABLE METALLIC ALLOYS. Applicant: KUMTA, PRASHANT N. The sequence listing filed with the application follows.

SEQUENCE LISTING (13 sequences)

SEQ ID NO: 1 - DNA, 19 bp, Artificial Sequence
  GAPDH Forward Primer
atggggaaggtgaaggtcg

SEQ ID NO: 2 - DNA, 20 bp, Artificial Sequence
  GAPDH Reverse Primer
taaaagcagccctggtgacc

SEQ ID NO: 3 - DNA, 19 bp, Artificial Sequence
  Alkaline phosphatase (ALPL) Forward Primer
gacccttgacccccacaat

SEQ ID NO: 4 - DNA, 20 bp, Artificial Sequence
  Alkaline Phosphatase (ALPL) Reverse Primer
gctcgtactgcatgtcccct

SEQ ID NO: 5 - DNA, 18 bp, Artificial Sequence
  Osteopontin (OPN) Forward Primer
ctcaggccagttgcagcc

SEQ ID NO: 6 - DNA, 24 bp, Artificial Sequence
  Osteopontin (OPN) Reverse Primer
caaaagcaaatcactgcaattctc

SEQ ID NO: 7 - DNA, 19 bp, Artificial Sequence
  GAPDH Forward Primer
ttgtcctgcgacttcaaca

SEQ ID NO: 8 - DNA, 22 bp, Artificial Sequence
  GAPDH Reverse Primer
gtggtccagggtttcttactcc

SEQ ID NO: 9 - DNA, 21 bp, Artificial Sequence
  RUNX2 Forward Primer
aacccacgaatgcactatcca

SEQ ID NO: 10 - DNA, 20 bp, Artificial Sequence
  RUNX2 Reverse Primer
cggacataccgagggacatg

SEQ ID NO: 11 - DNA, 18 bp, Artificial Sequence
  ALP Forward Primer
gacccttgacccccacaa

SEQ ID NO: 12 - DNA, 21 bp, Artificial Sequence
  Osteocalcin Forward Primer
ccggagcagtgtgagcttata

SEQ ID NO: 13 - DNA, 19 bp, Artificial Sequence
  Osteocalcin Reverse Primer
gatgcgtttgtaggcggtc